European Patent Application EP 4 813 408 A1, published September 30, 2026. Title: Chimeric antigen receptors comprising cytosolic CD4 costimulatory domain for immunotherapy. Applicant: Kemijski Institut. The sequence listing filed with the application follows.

SEQUENCE LISTING (45 sequences)

SEQ ID NO: 1 - DNA, 1473 bp, synthetic construct
  source 1..1473: mol_type = other DNA
gccctgcctgtgacagctctgctgctgcctctggccctgctgctgcatgccgccagacccgagcagaagctgatcagcgaggaggacctggacattcaaatgactcaaacaacttcatctttgtctgcaagcctgggagaccgcgtgacaataagctgccgagccagtcaagatatcagcaaatatctcaattggtatcagcaaaagcctgatgggactgttaaattgttgatataccatacgagtcgcctccacagcggagttccttctaggttttctggatcaggctccgggaccgactactccctcacgattagcaatcttgagcaggaggatatagccacatatttttgtcaacaaggaaacacacttccctacaccttcggtgggggaacgaaattggaaattactggtggcggcgggtctggaggtggcggtagtggaggcgggggctctgaagtcaagcttcaagaatcaggtccgggacttgtagcgccaagtcagtctctttccgtaacttgtaccgttagtggggtttccttgccagattacggagtaagttggattcgccaaccgcccagaaagggcttggaatggttgggtgttatctggggaagcgaaacaacatactataacagcgcactcaagtctcgcctcacgattattaaagataactctaaatctcaggtgttcctcaaaatgaactcattgcaaacggacgacactgccatctattactgtgcaaaacactattactacggcggctcttacgctatggattactggggccagggaacttcagtgacagtttctagtacaaccacccctgcccctagacctccaaccccagcccctacaatcgccagccagcctctgtctctgaggcccgaggcttgtagaccagctgctggcggagccgtgcacaccagaggactggatttcgcctgcgacatctacatctgggcccctctggccggcacatgtggcgtgctgctgctgagcctcgtgatcaccctgtactgccggtgcagacaccgcaggagacaagcagaaagactcagccaaataaagagactgctctctgagaagaagacatgccagtgtcctcacagattccagaaaacatgcagccccataagagtgaagttcagcagatccgccgacgcccctgcctaccagcagggacagaaccagctgtacaacgagctgaacctgggcagacgggaagagtacgacgtgctggacaagcggagaggccgggatcctgaaatgggcggcaagcccagacggaagaacccccaggaaggcctgtataacgaactgcagaaagacaagatggccgaggcctacagcgagatcggaatgaagggcgagcggagaagaggcaagggccacgatggcctgtaccagggcctgagcaccgccaccaaggacacctatgacgccctgcacatgcaggctttgccgcctaga

SEQ ID NO: 2 - DNA, 1599 bp, synthetic construct
  source 1..1599: mol_type = other DNA
gccctgcctgtgacagctctgctgctgcctctggccctgctgctgcatgccgccagacccgagcagaagctgatcagcgaggaggacctggacattcaaatgactcaaacaacttcatctttgtctgcaagcctgggagaccgcgtgacaataagctgccgagccagtcaagatatcagcaaatatctcaattggtatcagcaaaagcctgatgggactgttaaattgttgatataccatacgagtcgcctccacagcggagttccttctaggttttctggatcaggctccgggaccgactactccctcacgattagcaatcttgagcaggaggatatagccacatatttttgtcaacaaggaaacacacttccctacaccttcggtgggggaacgaaattggaaattactggtggcggcgggtctggaggtggcggtagtggaggcgggggctctgaagtcaagcttcaagaatcaggtccgggacttgtagcgccaagtcagtctctttccgtaacttgtaccgttagtggggtttccttgccagattacggagtaagttggattcgccaaccgcccagaaagggcttggaatggttgggtgttatctggggaagcgaaacaacatactataacagcgcactcaagtctcgcctcacgattattaaagataactctaaatctcaggtgttcctcaaaatgaactcattgcaaacggacgacactgccatctattactgtgcaaaacactattactacggcggctcttacgctatggattactggggccagggaacttcagtgacagtttctagtacaaccacccctgcccctagacctccaaccccagcccctacaatcgccagccagcctctgtctctgaggcccgaggcttgtagaccagctgctggcggagccgtgcacaccagaggactggatttcgcctgcgacatctacatctgggcccctctggccggcacatgtggcgtgctgctgctgagcctcgtgatcaccctgtactgccggtgcagacaccgcaggagacaagcagaaagactcagccaaataaagagactgctctctgagaagaagacatgccagtgtcctcacagattccagaaaacatgcagccccataaagcggggcagaaagaaactgctgtacatctttaagcagcccttcatgcggcccgtgcagaccacccaggaagaggacggctgctcctgcagattccccgaggaagaagaaggcggctgcgagctgagagtgaagttcagcagatccgccgacgcccctgcctaccagcagggacagaaccagctgtacaacgagctgaacctgggcagacgggaagagtacgacgtgctggacaagcggagaggccgggatcctgaaatgggcggcaagcccagacggaagaacccccaggaaggcctgtataacgaactgcagaaagacaagatggccgaggcctacagcgagatcggaatgaagggcgagcggagaagaggcaagggccacgatggcctgtaccagggcctgagcaccgccaccaaggacacctatgacgccctgcacatgcaggctttgccgcctaga

SEQ ID NO: 3 - DNA, 1599 bp, synthetic construct
  source 1..1599: mol_type = other DNA
gccctgcctgtgacagctctgctgctgcctctggccctgctgctgcatgccgccagacccgagcagaagctgatcagcgaggaggacctggacattcaaatgactcaaacaacttcatctttgtctgcaagcctgggagaccgcgtgacaataagctgccgagccagtcaagatatcagcaaatatctcaattggtatcagcaaaagcctgatgggactgttaaattgttgatataccatacgagtcgcctccacagcggagttccttctaggttttctggatcaggctccgggaccgactactccctcacgattagcaatcttgagcaggaggatatagccacatatttttgtcaacaaggaaacacacttccctacaccttcggtgggggaacgaaattggaaattactggtggcggcgggtctggaggtggcggtagtggaggcgggggctctgaagtcaagcttcaagaatcaggtccgggacttgtagcgccaagtcagtctctttccgtaacttgtaccgttagtggggtttccttgccagattacggagtaagttggattcgccaaccgcccagaaagggcttggaatggttgggtgttatctggggaagcgaaacaacatactataacagcgcactcaagtctcgcctcacgattattaaagataactctaaatctcaggtgttcctcaaaatgaactcattgcaaacggacgacactgccatctattactgtgcaaaacactattactacggcggctcttacgctatggattactggggccagggaacttcagtgacagtttctagtacaaccacccctgcccctagacctccaaccccagcccctacaatcgccagccagcctctgtctctgaggcccgaggcttgtagaccagctgctggcggagccgtgcacaccagaggactggatttcgcctgcgacatctacatctgggcccctctggccggcacatgtggcgtgctgctgctgagcctcgtgatcaccctgtactgcaagcggggcagaaagaaactgctgtacatctttaagcagcccttcatgcggcccgtgcagaccacccaggaagaggacggctgctcctgcagattccccgaggaagaagaaggcggctgcgagctgcggtgcagacaccgcaggagacaagcagaaagactcagccaaataaagagactgctctctgagaagaagacatgccagtgtcctcacagattccagaaaacatgcagccccataagagtgaagttcagcagatccgccgacgcccctgcctaccagcagggacagaaccagctgtacaacgagctgaacctgggcagacgggaagagtacgacgtgctggacaagcggagaggccgggatcctgaaatgggcggcaagcccagacggaagaacccccaggaaggcctgtataacgaactgcagaaagacaagatggccgaggcctacagcgagatcggaatgaagggcgagcggagaagaggcaagggccacgatggcctgtaccagggcctgagcaccgccaccaaggacacctatgacgccctgcacatgcaggctttgccgcctaga

SEQ ID NO: 4 - DNA, 1599 bp, synthetic construct
  source 1..1599: mol_type = other DNA
gccctgcctgtgacagctctgctgctgcctctggccctgctgctgcatgccgccagacccgagcagaagctgatcagcgaggaggacctggacattcaaatgactcaaacaacttcatctttgtctgcaagcctgggagaccgcgtgacaataagctgccgagccagtcaagatatcagcaaatatctcaattggtatcagcaaaagcctgatgggactgttaaattgttgatataccatacgagtcgcctccacagcggagttccttctaggttttctggatcaggctccgggaccgactactccctcacgattagcaatcttgagcaggaggatatagccacatatttttgtcaacaaggaaacacacttccctacaccttcggtgggggaacgaaattggaaattactggtggcggcgggtctggaggtggcggtagtggaggcgggggctctgaagtcaagcttcaagaatcaggtccgggacttgtagcgccaagtcagtctctttccgtaacttgtaccgttagtggggtttccttgccagattacggagtaagttggattcgccaaccgcccagaaagggcttggaatggttgggtgttatctggggaagcgaaacaacatactataacagcgcactcaagtctcgcctcacgattattaaagataactctaaatctcaggtgttcctcaaaatgaactcattgcaaacggacgacactgccatctattactgtgcaaaacactattactacggcggctcttacgctatggattactggggccagggaacttcagtgacagtttctagtacaaccacccctgcccctagacctccaaccccagcccctacaatcgccagccagcctctgtctctgaggcccgaggcttgtagaccagctgctggcggagccgtgcacaccagaggactggatttcgcctgcgacatctacatctgggcccctctggccggcacatgtggcgtgctgctgctgagcctcgtgatcaccctgtactgcaagcggggcagaaagaaactgctgtacatctttaagcagcccttcatgcggcccgtgcagaccacccaggaagaggacggctgctcctgcagattccccgaggaagaagaaggcggctgcgagctgagagtgaagttcagcagatccgccgacgcccctgcctaccagcagggacagaaccagctgtacaacgagctgaacctgggcagacgggaagagtacgacgtgctggacaagcggagaggccgggatcctgaaatgggcggcaagcccagacggaagaacccccaggaaggcctgtataacgaactgcagaaagacaagatggccgaggcctacagcgagatcggaatgaagggcgagcggagaagaggcaagggccacgatggcctgtaccagggcctgagcaccgccaccaaggacacctatgacgccctgcacatgcaggctttgccgcctagacggtgcagacaccgcaggagacaagcagaaagactcagccaaataaagagactgctctctgagaagaagacatgccagtgtcctcacagattccagaaaacatgcagccccata

SEQ ID NO: 5 - DNA, 60 bp, Homo sapiens
  source 1..60: mol_type = other DNA
gccctgcctgtgacagctctgctgctgcctctggccctgctgctgcatgccgccagaccc

SEQ ID NO: 6 - protein, 20 aa, Homo sapiens
ALPVTALLLPLALLLHAARP

SEQ ID NO: 7 - DNA, 30 bp, synthetic construct
  source 1..30: mol_type = other DNA
gagcagaagctgatcagcgaggaggacctg

SEQ ID NO: 8 - protein, 10 aa, synthetic construct
EQKLISEEDL

SEQ ID NO: 9 - DNA, 726 bp, synthetic construct
  source 1..726: mol_type = other DNA
gacattcaaatgactcaaacaacttcatctttgtctgcaagcctgggagaccgcgtgacaataagctgccgagccagtcaagatatcagcaaatatctcaattggtatcagcaaaagcctgatgggactgttaaattgttgatataccatacgagtcgcctccacagcggagttccttctaggttttctggatcaggctccgggaccgactactccctcacgattagcaatcttgagcaggaggatatagccacatatttttgtcaacaaggaaacacacttccctacaccttcggtgggggaacgaaattggaaattactggtggcggcgggtctggaggtggcggtagtggaggcgggggctctgaagtcaagcttcaagaatcaggtccgggacttgtagcgccaagtcagtctctttccgtaacttgtaccgttagtggggtttccttgccagattacggagtaagttggattcgccaaccgcccagaaagggcttggaatggttgggtgttatctggggaagcgaaacaacatactataacagcgcactcaagtctcgcctcacgattattaaagataactctaaatctcaggtgttcctcaaaatgaactcattgcaaacggacgacactgccatctattactgtgcaaaacactattactacggcggctcttacgctatggattactggggccagggaacttcagtgacagtttctagt

SEQ ID NO: 10 - protein, 242 aa, synthetic construct
DIQMTQTTSSLSASLGDRVTISCRASQDISKYLNWYQQKPDGTVKLLIYHTSRLHSGVPSRFSGSGSGTDYSLTISNLEQEDIATYFCQQGNTLPYTFGGGTKLEITGGGGSGGGGSGGGGSEVKLQESGPGLVAPSQSLSVTCTVSGVSLPDYGVSWIRQPPRKGLEWLGVIWGSETTYYNSALKSRLTIIKDNSKSQVFLKMNSLQTDDTAIYYCAKHYYYGGSYAMDYWGQGTSVTVSS

SEQ ID NO: 11 - DNA, 732 bp, synthetic construct
  source 1..732: mol_type = other DNA
gacatccagatgacccagagtcccagcagtctgagcgctagtgtaggcgaccgcgttaccatcacatgcagagcatctcaagatgtgaatacagcagttgcgtggtatcaacagaaacctggtaaagcccctaaactgctcatctatagtgcgtcctttctgtatagtggcgtcccctcacgcttcagcggctcacgctctgggacagactttaccttgaccatctcttcccttcagcctgaggactttgccacctattattgtcagcaacattacaccacaccaccaacattcgggcaggggacgaaagtagagataaaaaggacgggctctacaagtgggtctggaaaaccgggctcaggggaaggatctgaggtgcaactcgttgaaagtggcggcggattggtccagccggggggatccttgcgccttagctgtgctgcatcaggatttaatatcaaggacacttacatccactgggtaaggcaagcccctggaaaggggcttgagtgggtagcccggatctaccctacaaacggttatacccgctacgcggacagcgtgaaaggccgcttcacaatttcagccgatacttctaaaaacactgcgtacctccaaatgaactcactgcgggcggaagatactgcagtttattactgtagcagatggggtggggatgggttttatgccatggatgtatgggggcagggaacacttgtaaccgtttctagc

SEQ ID NO: 12 - protein, 244 aa, synthetic construct
DIQMTQSPSSLSASVGDRVTITCRASQDVNTAVAWYQQKPGKAPKLLIYSASFLYSGVPSRFSGSRSGTDFTLTISSLQPEDFATYYCQQHYTTPPTFGQGTKVEIKRTGSTSGSGKPGSGEGSEVQLVESGGGLVQPGGSLRLSCAASGFNIKDTYIHWVRQAPGKGLEWVARIYPTNGYTRYADSVKGRFTISADTSKNTAYLQMNSLRAEDTAVYYCSRWGGDGFYAMDVWGQGTLVTVSS

SEQ ID NO: 13 - DNA, 720 bp, synthetic construct
  source 1..720: mol_type = other DNA
caggtgcagctggtgcagagcggcgcggaagtgaaaaaaccgggcagcagcgtgaaagtgagctgcaaagcgagcggctatacctttaccagctatgtgatgcattgggtgcgccaggcgccgggccagggcctggaatggatgggctatattattccgtataacgatgcgaccaaatataacgaaaaatttaaaggccgcgtgaccattaccgcggataaaagcaccagcaccgcgtatatggaactgagcagcctgcgcagcgaagataccgcggtgtattattgcgcgcgctataactatgatggctattttgatgtgtggggccagggcaccctggtgaccgtgagcagcggtggcggcgggtctggaggtggcggtagtggaggcgggggctctgaaattgtgctgacccagagcccggcgaccctgagcctgagcccgggcgaacgcgcgaccctgagctgccgcgcgagccagagcattagcgattatctgcattggtatcagcagaaaccgggccaggcgccgcgcctgctgatttattatgcgagccagagcattaccggcattccggcgcgctttagcggcagcggcagcggcaccgattttaccctgaccattagcagcctggaaccggaagattttgcggtgtattattgccagaacggccatagctttccgccgacctttggcggcggcaccaaagtggaaattaaa

SEQ ID NO: 14 - protein, 240 aa, synthetic construct
QVQLVQSGAEVKKPGSSVKVSCKASGYTFTSYVMHWVRQAPGQGLEWMGYIIPYNDATKYNEKFKGRVTITADKSTSTAYMELSSLRSEDTAVYYCARYNYDGYFDVWGQGTLVTVSSGGGGSGGGGSGGGGSEIVLTQSPATLSLSPGERATLSCRASQSISDYLHWYQQKPGQAPRLLIYYASQSITGIPARFSGSGSGTDFTLTISSLEPEDFAVYYCQNGHSFPPTFGGGTKVEIK

SEQ ID NO: 15 - protein, 12 aa, synthetic construct
GGGSGGGSGGGS

SEQ ID NO: 16 - DNA, 141 bp, Homo sapiens
  source 1..141: mol_type = other DNA
acaaccacccctgcccctagacctccaaccccagcccctacaatcgccagccagcctctgtctctgaggcccgaggcttgtagaccagctgctggcggagccgtgcacaccagaggactggatttcgcctgcgacatctac

SEQ ID NO: 17 - protein, 47 aa, Homo sapiens
TTTPAPRPPTPAPTIASQPLSLRPEACRPAAGGAVHTRGLDFACDIY

SEQ ID NO: 18 - DNA, 66 bp, Homo sapiens
  source 1..66: mol_type = other DNA
atctgggcccctctggccggcacatgtggcgtgctgctgctgagcctcgtgatcaccctgtactgc

SEQ ID NO: 19 - protein, 22 aa, Homo sapiens
IWAPLAGTCGVLLLSLVITLYC

SEQ ID NO: 20 - DNA, 114 bp, Homo sapiens
  source 1..114: mol_type = other DNA
cggtgcagacaccgcaggagacaagcagaaagactcagccaaataaagagactgctctctgagaagaagacatgccagtgtcctcacagattccagaaaacatgcagccccata

SEQ ID NO: 21 - protein, 38 aa, Homo sapiens
RCRHRRRQAERLSQIKRLLSEKKTCQCPHRFQKTCSPI

SEQ ID NO: 22 - DNA, 126 bp, Homo sapiens
  source 1..126: mol_type = other DNA
aagcggggcagaaagaaactgctgtacatctttaagcagcccttcatgcggcccgtgcagaccacccaggaagaggacggctgctcctgcagattccccgaggaagaagaaggcggctgcgagctg

SEQ ID NO: 23 - protein, 42 aa, Homo sapiens
KRGRKKLLYIFKQPFMRPVQTTQEEDGCSCRFPEEEEGGCEL

SEQ ID NO: 24 - DNA, 336 bp, Homo sapiens
  source 1..336: mol_type = other DNA
agagtgaagttcagcagatccgccgacgcccctgcctaccagcagggacagaaccagctgtacaacgagctgaacctgggcagacgggaagagtacgacgtgctggacaagcggagaggccgggatcctgaaatgggcggcaagcccagacggaagaacccccaggaaggcctgtataacgaactgcagaaagacaagatggccgaggcctacagcgagatcggaatgaagggcgagcggagaagaggcaagggccacgatggcctgtaccagggcctgagcaccgccaccaaggacacctatgacgccctgcacatgcaggctttgccgcctaga

SEQ ID NO: 25 - protein, 112 aa, Homo sapiens
RVKFSRSADAPAYQQGQNQLYNELNLGRREEYDVLDKRRGRDPEMGGKPRRKNPQEGLYNELQKDKMAEAYSEIGMKGERRRGKGHDGLYQGLSTATKDTYDALHMQALPPR

SEQ ID NO: 26 - protein, 458 aa, Homo sapiens
MNRGVPFRHLLLVLQLALLPAATQGKKVVLGKKGDTVELTCTASQKKSIQFHWKNSNQIKILGNQGSFLTKGPSKLNDRADSRRSLWDQGNFPLIIKNLKIEDSDTYICEVEDQKEEVQLLVFGLTANSDTHLLQGQSLTLTLESPPGSSPSVQCRSPRGKNIQGGKTLSVSQLELQDSGTWTCTVLQNQKKVEFKIDIVVLAFQKASSIVYKKEGEQVEFSFPLAFTVEKLTGSGELWWQAERASSSKSWITFDLKNKEVSVKRVTQDPKLQMGKKLPLHLTLPQALPQYAGSGNLTLALEAKTGKLHQEVNLVVMRATQLQKNLTCEVWGPTSPKLMLSLKLENKEAKVSKREKAVWVLNPEAGMWQCLLSDSGQVLLESNIKVLPTWSTPVQPMALIVLGGVAGLLLFIGLGIFFCVRCRHRRRQAERMSQIKRLLSEKKTCQCPHRFQKTCSPI

SEQ ID NO: 27 - protein, 38 aa, Homo sapiens
RCRHRRRQAERMSQIKRLLSEKKTCQCPHRFQKTCSPI

SEQ ID NO: 28 - protein, 491 aa, synthetic construct
ALPVTALLLPLALLLHAARPEQKLISEEDLDIQMTQTTSSLSASLGDRVTISCRASQDISKYLNWYQQKPDGTVKLLIYHTSRLHSGVPSRFSGSGSGTDYSLTISNLEQEDIATYFCQQGNTLPYTFGGGTKLEITGGGGSGGGGSGGGGSEVKLQESGPGLVAPSQSLSVTCTVSGVSLPDYGVSWIRQPPRKGLEWLGVIWGSETTYYNSALKSRLTIIKDNSKSQVFLKMNSLQTDDTAIYYCAKHYYYGGSYAMDYWGQGTSVTVSSTTTPAPRPPTPAPTIASQPLSLRPEACRPAAGGAVHTRGLDFACDIYIWAPLAGTCGVLLLSLVITLYCRCRHRRRQAERLSQIKRLLSEKKTCQCPHRFQKTCSPIRVKFSRSADAPAYQQGQNQLYNELNLGRREEYDVLDKRRGRDPEMGGKPRRKNPQEGLYNELQKDKMAEAYSEIGMKGERRRGKGHDGLYQGLSTATKDTYDALHMQALPPR

SEQ ID NO: 29 - protein, 533 aa, synthetic construct
ALPVTALLLPLALLLHAARPEQKLISEEDLDIQMTQTTSSLSASLGDRVTISCRASQDISKYLNWYQQKPDGTVKLLIYHTSRLHSGVPSRFSGSGSGTDYSLTISNLEQEDIATYFCQQGNTLPYTFGGGTKLEITGGGGSGGGGSGGGGSEVKLQESGPGLVAPSQSLSVTCTVSGVSLPDYGVSWIRQPPRKGLEWLGVIWGSETTYYNSALKSRLTIIKDNSKSQVFLKMNSLQTDDTAIYYCAKHYYYGGSYAMDYWGQGTSVTVSSTTTPAPRPPTPAPTIASQPLSLRPEACRPAAGGAVHTRGLDFACDIYIWAPLAGTCGVLLLSLVITLYCRCRHRRRQAERLSQIKRLLSEKKTCQCPHRFQKTCSPIKRGRKKLLYIFKQPFMRPVQTTQEEDGCSCRFPEEEEGGCELRVKFSRSADAPAYQQGQNQLYNELNLGRREEYDVLDKRRGRDPEMGGKPRRKNPQEGLYNELQKDKMAEAYSEIGMKGERRRGKGHDGLYQGLSTATKDTYDALHMQALPPR

SEQ ID NO: 30 - protein, 533 aa, synthetic construct
ALPVTALLLPLALLLHAARPEQKLISEEDLDIQMTQTTSSLSASLGDRVTISCRASQDISKYLNWYQQKPDGTVKLLIYHTSRLHSGVPSRFSGSGSGTDYSLTISNLEQEDIATYFCQQGNTLPYTFGGGTKLEITGGGGSGGGGSGGGGSEVKLQESGPGLVAPSQSLSVTCTVSGVSLPDYGVSWIRQPPRKGLEWLGVIWGSETTYYNSALKSRLTIIKDNSKSQVFLKMNSLQTDDTAIYYCAKHYYYGGSYAMDYWGQGTSVTVSSTTTPAPRPPTPAPTIASQPLSLRPEACRPAAGGAVHTRGLDFACDIYIWAPLAGTCGVLLLSLVITLYCKRGRKKLLYIFKQPFMRPVQTTQEEDGCSCRFPEEEEGGCELRCRHRRRQAERLSQIKRLLSEKKTCQCPHRFQKTCSPIRVKFSRSADAPAYQQGQNQLYNELNLGRREEYDVLDKRRGRDPEMGGKPRRKNPQEGLYNELQKDKMAEAYSEIGMKGERRRGKGHDGLYQGLSTATKDTYDALHMQALPPR

SEQ ID NO: 31 - protein, 533 aa, synthetic construct
ALPVTALLLPLALLLHAARPEQKLISEEDLDIQMTQTTSSLSASLGDRVTISCRASQDISKYLNWYQQKPDGTVKLLIYHTSRLHSGVPSRFSGSGSGTDYSLTISNLEQEDIATYFCQQGNTLPYTFGGGTKLEITGGGGSGGGGSGGGGSEVKLQESGPGLVAPSQSLSVTCTVSGVSLPDYGVSWIRQPPRKGLEWLGVIWGSETTYYNSALKSRLTIIKDNSKSQVFLKMNSLQTDDTAIYYCAKHYYYGGSYAMDYWGQGTSVTVSSTTTPAPRPPTPAPTIASQPLSLRPEACRPAAGGAVHTRGLDFACDIYIWAPLAGTCGVLLLSLVITLYCRCRHRRRQAERLSQIKRLLSEKKTCQCPHRFQKTCSPIRVKFSRSADAPAYQQGQNQLYNELNLGRREEYDVLDKRRGRDPEMGGKPRRKNPQEGLYNELQKDKMAEAYSEIGMKGERRRGKGHDGLYQGLSTATKDTYDALHMQALPPRKRGRKKLLYIFKQPFMRPVQTTQEEDGCSCRFPEEEEGGCEL

SEQ ID NO: 32 - protein, 493 aa, synthetic construct
ALPVTALLLPLALLLHAARPEQKLISEEDLDIQMTQSPSSLSASVGDRVTITCRASQDVNTAVAWYQQKPGKAPKLLIYSASFLYSGVPSRFSGSRSGTDFTLTISSLQPEDFATYYCQQHYTTPPTFGQGTKVEIKRTGSTSGSGKPGSGEGSEVQLVESGGGLVQPGGSLRLSCAASGFNIKDTYIHWVRQAPGKGLEWVARIYPTNGYTRYADSVKGRFTISADTSKNTAYLQMNSLRAEDTAVYYCSRWGGDGFYAMDVWGQGTLVTVSSTTTPAPRPPTPAPTIASQPLSLRPEACRPAAGGAVHTRGLDFACDIYIWAPLAGTCGVLLLSLVITLYCRCRHRRRQAERLSQIKRLLSEKKTCQCPHRFQKTCSPIRVKFSRSADAPAYQQGQNQLYNELNLGRREEYDVLDKRRGRDPEMGGKPRRKNPQEGLYNELQKDKMAEAYSEIGMKGERRRGKGHDGLYQGLSTATKDTYDALHMQALPPR

SEQ ID NO: 33 - protein, 535 aa, synthetic construct
ALPVTALLLPLALLLHAARPEQKLISEEDLDIQMTQSPSSLSASVGDRVTITCRASQDVNTAVAWYQQKPGKAPKLLIYSASFLYSGVPSRFSGSRSGTDFTLTISSLQPEDFATYYCQQHYTTPPTFGQGTKVEIKRTGSTSGSGKPGSGEGSEVQLVESGGGLVQPGGSLRLSCAASGFNIKDTYIHWVRQAPGKGLEWVARIYPTNGYTRYADSVKGRFTISADTSKNTAYLQMNSLRAEDTAVYYCSRWGGDGFYAMDVWGQGTLVTVSSTTTPAPRPPTPAPTIASQPLSLRPEACRPAAGGAVHTRGLDFACDIYIWAPLAGTCGVLLLSLVITLYCRCRHRRRQAERLSQIKRLLSEKKTCQCPHRFQKTCSPIKRGRKKLLYIFKQPFMRPVQTTQEEDGCSCRFPEEEEGGCELRVKFSRSADAPAYQQGQNQLYNELNLGRREEYDVLDKRRGRDPEMGGKPRRKNPQEGLYNELQKDKMAEAYSEIGMKGERRRGKGHDGLYQGLSTATKDTYDALHMQALPPR

SEQ ID NO: 34 - protein, 535 aa, synthetic construct
ALPVTALLLPLALLLHAARPEQKLISEEDLDIQMTQSPSSLSASVGDRVTITCRASQDVNTAVAWYQQKPGKAPKLLIYSASFLYSGVPSRFSGSRSGTDFTLTISSLQPEDFATYYCQQHYTTPPTFGQGTKVEIKRTGSTSGSGKPGSGEGSEVQLVESGGGLVQPGGSLRLSCAASGFNIKDTYIHWVRQAPGKGLEWVARIYPTNGYTRYADSVKGRFTISADTSKNTAYLQMNSLRAEDTAVYYCSRWGGDGFYAMDVWGQGTLVTVSSTTTPAPRPPTPAPTIASQPLSLRPEACRPAAGGAVHTRGLDFACDIYIWAPLAGTCGVLLLSLVITLYCKRGRKKLLYIFKQPFMRPVQTTQEEDGCSCRFPEEEEGGCELRCRHRRRQAERLSQIKRLLSEKKTCQCPHRFQKTCSPIRVKFSRSADAPAYQQGQNQLYNELNLGRREEYDVLDKRRGRDPEMGGKPRRKNPQEGLYNELQKDKMAEAYSEIGMKGERRRGKGHDGLYQGLSTATKDTYDALHMQALPPR

SEQ ID NO: 35 - protein, 535 aa, synthetic construct
ALPVTALLLPLALLLHAARPEQKLISEEDLDIQMTQSPSSLSASVGDRVTITCRASQDVNTAVAWYQQKPGKAPKLLIYSASFLYSGVPSRFSGSRSGTDFTLTISSLQPEDFATYYCQQHYTTPPTFGQGTKVEIKRTGSTSGSGKPGSGEGSEVQLVESGGGLVQPGGSLRLSCAASGFNIKDTYIHWVRQAPGKGLEWVARIYPTNGYTRYADSVKGRFTISADTSKNTAYLQMNSLRAEDTAVYYCSRWGGDGFYAMDVWGQGTLVTVSSTTTPAPRPPTPAPTIASQPLSLRPEACRPAAGGAVHTRGLDFACDIYIWAPLAGTCGVLLLSLVITLYCRCRHRRRQAERLSQIKRLLSEKKTCQCPHRFQKTCSPIRVKFSRSADAPAYQQGQNQLYNELNLGRREEYDVLDKRRGRDPEMGGKPRRKNPQEGLYNELQKDKMAEAYSEIGMKGERRRGKGHDGLYQGLSTATKDTYDALHMQALPPRKRGRKKLLYIFKQPFMRPVQTTQEEDGCSCRFPEEEEGGCEL

SEQ ID NO: 36 - protein, 489 aa, synthetic construct
ALPVTALLLPLALLLHAARPEQKLISEEDLQVQLVQSGAEVKKPGSSVKVSCKASGYTFTSYVMHWVRQAPGQGLEWMGYIIPYNDATKYNEKFKGRVTITADKSTSTAYMELSSLRSEDTAVYYCARYNYDGYFDVWGQGTLVTVSSGGGGSGGGGSGGGGSEIVLTQSPATLSLSPGERATLSCRASQSISDYLHWYQQKPGQAPRLLIYYASQSITGIPARFSGSGSGTDFTLTISSLEPEDFAVYYCQNGHSFPPTFGGGTKVEIKTTTPAPRPPTPAPTIASQPLSLRPEACRPAAGGAVHTRGLDFACDIYIWAPLAGTCGVLLLSLVITLYCRCRHRRRQAERLSQIKRLLSEKKTCQCPHRFQKTCSPIRVKFSRSADAPAYQQGQNQLYNELNLGRREEYDVLDKRRGRDPEMGGKPRRKNPQEGLYNELQKDKMAEAYSEIGMKGERRRGKGHDGLYQGLSTATKDTYDALHMQALPPR

SEQ ID NO: 37 - protein, 531 aa, synthetic construct
ALPVTALLLPLALLLHAARPEQKLISEEDLQVQLVQSGAEVKKPGSSVKVSCKASGYTFTSYVMHWVRQAPGQGLEWMGYIIPYNDATKYNEKFKGRVTITADKSTSTAYMELSSLRSEDTAVYYCARYNYDGYFDVWGQGTLVTVSSGGGGSGGGGSGGGGSEIVLTQSPATLSLSPGERATLSCRASQSISDYLHWYQQKPGQAPRLLIYYASQSITGIPARFSGSGSGTDFTLTISSLEPEDFAVYYCQNGHSFPPTFGGGTKVEIKTTTPAPRPPTPAPTIASQPLSLRPEACRPAAGGAVHTRGLDFACDIYIWAPLAGTCGVLLLSLVITLYCRCRHRRRQAERLSQIKRLLSEKKTCQCPHRFQKTCSPIKRGRKKLLYIFKQPFMRPVQTTQEEDGCSCRFPEEEEGGCELRVKFSRSADAPAYQQGQNQLYNELNLGRREEYDVLDKRRGRDPEMGGKPRRKNPQEGLYNELQKDKMAEAYSEIGMKGERRRGKGHDGLYQGLSTATKDTYDALHMQALPPR

SEQ ID NO: 38 - protein, 531 aa, synthetic construct
ALPVTALLLPLALLLHAARPEQKLISEEDLQVQLVQSGAEVKKPGSSVKVSCKASGYTFTSYVMHWVRQAPGQGLEWMGYIIPYNDATKYNEKFKGRVTITADKSTSTAYMELSSLRSEDTAVYYCARYNYDGYFDVWGQGTLVTVSSGGGGSGGGGSGGGGSEIVLTQSPATLSLSPGERATLSCRASQSISDYLHWYQQKPGQAPRLLIYYASQSITGIPARFSGSGSGTDFTLTISSLEPEDFAVYYCQNGHSFPPTFGGGTKVEIKTTTPAPRPPTPAPTIASQPLSLRPEACRPAAGGAVHTRGLDFACDIYIWAPLAGTCGVLLLSLVITLYCKRGRKKLLYIFKQPFMRPVQTTQEEDGCSCRFPEEEEGGCELRCRHRRRQAERLSQIKRLLSEKKTCQCPHRFQKTCSPIRVKFSRSADAPAYQQGQNQLYNELNLGRREEYDVLDKRRGRDPEMGGKPRRKNPQEGLYNELQKDKMAEAYSEIGMKGERRRGKGHDGLYQGLSTATKDTYDALHMQALPPR

SEQ ID NO: 39 - protein, 530 aa, synthetic construct
ALPVTALLLPLALLLHAARPEQKLISEEDLQVQLVQSGAEVKKPGSSVKVSCKASGYTFTSYVMHWVRQAPGQGLEWMGYIIPYNDATKYNEKFKGRVTITADKSTSTAYMELSSLRSEDTAVYYCARYNYDGYFDVWGQGTLVTVSSGGGGSGGGGSGGGGSEIVLTQSPALSLSPGERATLSCRASQSISDYLHWYQQKPGQAPRLLIYYASQSITGIPARFSGSGSGTDFTLTISSLEPEDFAVYYCQNGHSFPPTFGGGTKVEIKTTTPAPRPPTPAPTIASQPLSLRPEACRPAAGGAVHTRGLDFACDIYIWAPLAGTCGVLLLSLVITLYCRCRHRRRQAERLSQIKRLLSEKKTCQCPHRFQKTCSPIRVKFSRSADAPAYQQGQNQLYNELNLGRREEYDVLDKRRGRDPEMGGKPRRKNPQEGLYNELQKDKMAEAYSEIGMKGERRRGKGHDGLYQGLSTATKDTYDALHMQALPPRKRGRKKLLYIFKQPFMRPVQTTQEEDGCSCRFPEEEEGGCEL

SEQ ID NO: 40 - DNA, 729 bp, synthetic construct
  source 1..729: mol_type = other DNA
gacgtcgtcatgacgcaaactccgctctccctcccagtatctttgggagaccaggcgagtatttcatgtcgaagcagccaaagtttggtgcatcgcaacggaaatacgtacctgcactggtatcttcaaaagccgggccagagccctaaacttctgattcacaaggttagtaaccgattttctggtgtgcctgaccgcttctctgggtcaggctccggtacggactttacgctcaaaataagccgggtcgaggccgaagacctgggcgtctatttttgctctcagtcaactcatgttcctccgttgacatttggggcaggcactaaattggaactcaagagagcgggcggaggcggatctgggggaggaggcagtggaggcggagggtctgaagtgcaattgctgcaaagtgggccagagttggaaaagcctggagcttccgtaatgatttcctgtaaggcctcaggaagctcctttaccggatataatatgaattgggtacgacagaacatcggtaaaagtcttgaatggatcggtgcaatcgacccgtactacggaggtactagttataaccaaaaattcaaaggtcgcgccactcttactgtcgataagtcctctagcacagcctatatgcacctcaagagcctgacgtcagaagactcagccgtatactattgcgtgagcggtatggagtattggggccaagggacatctgtaactgtctctagc

SEQ ID NO: 41 - protein, 243 aa, synthetic construct
DVVMTQTPLSLPVSLGDQASISCRSSQSLVHRNGNTYLHWYLQKPGQSPKLLIHKVSNRFSGVPDRFSGSGSGTDFTLKISRVEAEDLGVYFCSQSTHVPPLTFGAGTKLELKRAGGGGSGGGGSGGGGSEVQLLQSGPELEKPGASVMISCKASGSSFTGYNMNWVRQNIGKSLEWIGAIDPYYGGTSYNQKFKGRATLTVDKSSSTAYMHLKSLTSEDSAVYYCVSGMEYWGQGTSVTVSS

SEQ ID NO: 42 - protein, 492 aa, synthetic construct
ALPVTALLLPLALLLHAARPEQKLISEEDLDVVMTQTPLSLPVSLGDQASISCRSSQSLVHRNGNTYLHWYLQKPGQSPKLLIHKVSNRFSGVPDRFSGSGSGTDFTLKISRVEAEDLGVYFCSQSTHVPPLTFGAGTKLELKRAGGGGSGGGGSGGGGSEVQLLQSGPELEKPGASVMISCKASGSSFTGYNMNWVRQNIGKSLEWIGAIDPYYGGTSYNQKFKGRATLTVDKSSSTAYMHLKSLTSEDSAVYYCVSGMEYWGQGTSVTVSSTTTPAPRPPTPAPTIASQPLSLRPEACRPAAGGAVHTRGLDFACDIYIWAPLAGTCGVLLLSLVITLYCRCRHRRRQAERLSQIKRLLSEKKTCQCPHRFQKTCSPIRVKFSRSADAPAYQQGQNQLYNELNLGRREEYDVLDKRRGRDPEMGGKPRRKNPQEGLYNELQKDKMAEAYSEIGMKGERRRGKGHDGLYQGLSTATKDTYDALHMQALPPR

SEQ ID NO: 43 - protein, 534 aa, synthetic construct
ALPVTALLLPLALLLHAARPEQKLISEEDLDVVMTQTPLSLPVSLGDQASISCRSSQSLVHRNGNTYLHWYLQKPGQSPKLLIHKVSNRFSGVPDRFSGSGSGTDFTLKISRVEAEDLGVYFCSQSTHVPPLTFGAGTKLELKRAGGGGSGGGGSGGGGSEVQLLQSGPELEKPGASVMISCKASGSSFTGYNMNWVRQNIGKSLEWIGAIDPYYGGTSYNQKFKGRATLTVDKSSSTAYMHLKSLTSEDSAVYYCVSGMEYWGQGTSVTVSSTTTPAPRPPTPAPTIASQPLSLRPEACRPAAGGAVHTRGLDFACDIYIWAPLAGTCGVLLLSLVITLYCRCRHRRRQAERLSQIKRLLSEKKTCQCPHRFQKTCSPIKRGRKKLLYIFKQPFMRPVQTTQEEDGCSCRFPEEEEGGCELRVKFSRSADAPAYQQGQNQLYNELNLGRREEYDVLDKRRGRDPEMGGKPRRKNPQEGLYNELQKDKMAEAYSEIGMKGERRRGKGHDGLYQGLSTATKDTYDALHMQALPPR

SEQ ID NO: 44 - protein, 534 aa, synthetic construct
ALPVTALLLPLALLLHAARPEQKLISEEDLDVVMTQTPLSLPVSLGDQASISCRSSQSLVHRNGNTYLHWYLQKPGQSPKLLIHKVSNRFSGVPDRFSGSGSGTDFTLKISRVEAEDLGVYFCSQSTHVPPLTFGAGTKLELKRAGGGGSGGGGSGGGGSEVQLLQSGPELEKPGASVMISCKASGSSFTGYNMNWVRQNIGKSLEWIGAIDPYYGGTSYNQKFKGRATLTVDKSSSTAYMHLKSLTSEDSAVYYCVSGMEYWGQGTSVTVSSTTTPAPRPPTPAPTIASQPLSLRPEACRPAAGGAVHTRGLDFACDIYIWAPLAGTCGVLLLSLVITLYCKRGRKKLLYIFKQPFMRPVQTTQEEDGCSCRFPEEEEGGCELRCRHRRRQAERLSQIKRLLSEKKTCQCPHRFQKTCSPIRVKFSRSADAPAYQQGQNQLYNELNLGRREEYDVLDKRRGRDPEMGGKPRRKNPQEGLYNELQKDKMAEAYSEIGMKGERRRGKGHDGLYQGLSTATKDTYDALHMQALPPR

SEQ ID NO: 45 - protein, 534 aa, synthetic construct
ALPVTALLLPLALLLHAARPEQKLISEEDLDVVMTQTPLSLPVSLGDQASISCRSSQSLVHRNGNTYLHWYLQKPGQSPKLLIHKVSNRFSGVPDRFSGSGSGTDFTLKISRVEAEDLGVYFCSQSTHVPPLTFGAGTKLELKRAGGGGSGGGGSGGGGSEVQLLQSGPELEKPGASVMISCKASGSSFTGYNMNWVRQNIGKSLEWIGAIDPYYGGTSYNQKFKGRATLTVDKSSSTAYMHLKSLTSEDSAVYYCVSGMEYWGQGTSVTVSSTTTPAPRPPTPAPTIASQPLSLRPEACRPAAGGAVHTRGLDFACDIYIWAPLAGTCGVLLLSLVITLYCRCRHRRRQAERLSQIKRLLSEKKTCQCPHRFQKTCSPIRVKFSRSADAPAYQQGQNQLYNELNLGRREEYDVLDKRRGRDPEMGGKPRRKNPQEGLYNELQKDKMAEAYSEIGMKGERRRGKGHDGLYQGLSTATKDTYDALHMQALPPRKRGRKKLLYIFKQPFMRPVQTTQEEDGCSCRFPEEEEGGCEL